European Patent Application EP 4 700 046 A1, published February 25, 2026. Title: Anti-CXCR2 antibody and use thereof. Applicant: Scripps Korea Antibody Institute. Application KR. The sequence listing filed with the application follows.

SEQUENCE LISTING (74 sequences)

SEQ ID NO: 1 - protein, 8 aa, synthetic construct
GFTFSNYS

SEQ ID NO: 2 - protein, 8 aa, synthetic construct
IYYNGGST

SEQ ID NO: 3 - protein, 20 aa, synthetic construct
ARGPRICEIRKCYSANAMDV

SEQ ID NO: 4 - protein, 8 aa, synthetic construct
SSNIGNNA

SEQ ID NO: 5 - skipped

SEQ ID NO: 6 - protein, 11 aa, synthetic construct
GTWDASLSAYV

SEQ ID NO: 7 - protein, 8 aa, synthetic construct
GFTFSNYA

SEQ ID NO: 8 - protein, 8 aa, synthetic construct
ISPSGSSK

SEQ ID NO: 9 - protein, 9 aa, synthetic construct
AKHNRHFDY

SEQ ID NO: 10 - protein, 8 aa, synthetic construct
SSNIGSHY

SEQ ID NO: 11 - skipped

SEQ ID NO: 12 - protein, 11 aa, synthetic construct
GSWDDSLNAYV

SEQ ID NO: 13 - protein, 8 aa, synthetic construct
GFTFSNYS

SEQ ID NO: 14 - protein, 8 aa, synthetic construct
ISSGGGSK

SEQ ID NO: 15 - protein, 9 aa, synthetic construct
ARQATAFDY

SEQ ID NO: 16 - protein, 8 aa, synthetic construct
SSNIGNNS

SEQ ID NO: 17 - skipped

SEQ ID NO: 18 - protein, 11 aa, synthetic construct
GTWDDSLSAYV

SEQ ID NO: 19 - protein, 8 aa, synthetic construct
GFTFSGYP

SEQ ID NO: 20 - protein, 8 aa, synthetic construct
ISSSGGNT

SEQ ID NO: 21 - protein, 20 aa, synthetic construct
ARFGIHHPDRALYYANAMDV

SEQ ID NO: 22 - protein, 8 aa, synthetic construct
SSNIGNND

SEQ ID NO: 23 - skipped

SEQ ID NO: 24 - protein, 11 aa, synthetic construct
ATWDASLSAYV

SEQ ID NO: 25 - protein, 116 aa, synthetic construct
EVQLLESGGGLVQPGGSLRLSCAASGFTFSNYAMSWVRQAPGKGLEWVSSISPSGSSKYYADSVKGRFTISRDNSKNTLYLQMNSLRAEDTAVYYCAKHNRHFDYWGQGTLVTVSS

SEQ ID NO: 26 - protein, 110 aa, synthetic construct
QSVLTQPPSASGTPGQRVTISCTGSSSNIGSHYVSWYQQLPGTAPKLLIYDNNHRPSGVPDRFSGSKSGTSASLAISGLRSEDEADYYCGSWDDSLNAYVFGGGTKLTVL

SEQ ID NO: 27 - protein, 127 aa, synthetic construct
EVQLLESGGGLVQPGGSLRLSCAASGFTFSGYPMSWVRQAPGKGLEWVSSISSSGGNTYYADSVKGRFTISRDNSKNTLYLQMNSLRAEDTAVYYCARFGIHHPDRALYYANAMDVWGQGTLVTVSS

SEQ ID NO: 28 - protein, 110 aa, synthetic construct
QSVLTQPPSASGTPGQRVTISCSGSSSNIGNNDVNWYQQLPGTAPKLLIYADNQRPSGVPDRFSGSKSGTSASLAISGLRSEDEADYYCATWDASLSAYVFGGGTKLTVL

SEQ ID NO: 29 - protein, 677 aa, synthetic construct
EVQLLESGGGLVQPGGSLRLSCAASGFTFSNYSMSWVRQAPGKGLEWVSWIYYNGGSTYYADSVKGRFTISRDNSKNTLYLQMNSLRAEDTAVYYCARGPRICEIRKCYSANAMDVWGQGTLVTVSSGPSSTKGPSVFPLAPSSKSTSGGTAALGCLVKDYFPEPVTVSWNSGALTSGVHTFPAVLQSSGLYSLSSVVTVPSSSLGTQTYICNVNHKPSNTKVDKKVEPKSCDKTHTCPPCPAPELLGGPSVFLFPPKPKDTLMISRTPEVTCVVVDVSHEDPEVKFNWYVDGVEVHNAKTKPREEQYNSTYRVVSVLTVLHQDWLNGKEYKCKVSNKALPAPIEKTISKAKGQPREPQVYTLPPSRDELTKNQVSLTCLVKGFYPSDIAVEWESNGQPENNYKTTPPVLDSDGSFFLYSKLTVDKSRWQQGNVFSCSVMHEALHNHYTQKSLSLSPGKQSVLTQPPSASGTPGQRVTISCSGSSSNIGNNAVSWYQQLPGTAPKLLIYANSNRPSGVPDRFSGSKSGTSASLAISGLRSEDEADYYCGTWDASLSAYVFGGGTKLTVLRTVAAPSVFIFPPSDEQLKSGTASVVCLLNNFYPREAKVQWKVDNALQSGNSQESVTEQDSKDSTYSLSSTLTLSKADYEKHKVYACEVTHQGLSSPVTKSFNRGECF

SEQ ID NO: 30 - protein, 666 aa, synthetic construct
EVQLLESGGGLVQPGGSLRLSCAASGFTFSNYAMSWVRQAPGKGLEWVSSISPSGSSKYYADSVKGRFTISRDNSKNTLYLQMNSLRAEDTAVYYCAKHNRHFDYWGQGTLVTVSSGPSSTKGPSVFPLAPSSKSTSGGTAALGCLVKDYFPEPVTVSWNSGALTSGVHTFPAVLQSSGLYSLSSVVTVPSSSLGTQTYICNVNHKPSNTKVDKKVEPKSCDKTHTCPPCPAPELLGGPSVFLFPPKPKDTLMISRTPEVTCVVVDVSHEDPEVKFNWYVDGVEVHNAKTKPREEQYNSTYRVVSVLTVLHQDWLNGKEYKCKVSNKALPAPIEKTISKAKGQPREPQVYTLPPSRDELTKNQVSLTCLVKGFYPSDIAVEWESNGQPENNYKTTPPVLDSDGSFFLYSKLTVDKSRWQQGNVFSCSVMHEALHNHYTQKSLSLSPGKQSVLTQPPSASGTPGQRVTISCTGSSSNIGSHYVSWYQQLPGTAPKLLIYDNNHRPSGVPDRFSGSKSGTSASLAISGLRSEDEADYYCGSWDDSLNAYVFGGGTKLTVLRTVAAPSVFIFPPSDEQLKSGTASVVCLLNNFYPREAKVQWKVDNALQSGNSQESVTEQDSKDSTYSLSSTLTLSKADYEKHKVYACEVTHQGLSSPVTKSFNRGECF

SEQ ID NO: 31 - protein, 666 aa, synthetic construct
EVQLLESGEGLVQPGGSLRLSCAASGFTFSNYSMSWVRQAPGKGLEWVSGISSGGGSKYYADSVKGRFTISRDNSKNTLYLQMNSLRAEDTAVYYCARQATAFDYWGQGTLVTVSSGPSSTKGPSVFPLAPSSKSTSGGTAALGCLVKDYFPEPVTVSWNSGALTSGVHTFPAVLQSSGLYSLSSVVTVPSSSLGTQTYICNVNHKPSNTKVDKKVEPKSCDKTHTCPPCPAPELLGGPSVFLFPPKPKDTLMISRTPEVTCVVVDVSHEDPEVKFNWYVDGVEVHNAKTKPREEQYNSTYRVVSVLTVLHQDWLNGKEYKCKVSNKALPAPIEKTISKAKGQPREPQVYTLPPSRDELTKNQVSLTCLVKGFYPSDIAVEWESNGQPENNYKTTPPVLDSDGSFFLYSKLTVDKSRWQQGNVFSCSVMHEALHNHYTQKSLSLSPGKQSVLTQPPSASGTPGQRVTISCTGSSSNIGNNSVTWYQQLPGTAPKLLIYSDSNRPSGVPDRFSGSKSGTSASLAISGLRSEDEADYYCGTWDDSLSAYVFGGGTKLTVLRTVAAPSVFIFPPSDEQLKSGTASVVCLLNNFYPREAKVQWKVDNALQSGNSQESVTEQDSKDSTYSLSSTLTLSKADYEKHKVYACEVTHQGLSSPVTKSFNRGECF

SEQ ID NO: 32 - protein, 677 aa, synthetic construct
EVQLLESGGGLVQPGGSLRLSCAASGFTFSGYPMSWVRQAPGKGLEWVSSISSSGGNTYYADSVKGRFTISRDNSKNTLYLQMNSLRAEDTAVYYCARFGIHHPDRALYYANAMDVWGQGTLVTVSSGPSSTKGPSVFPLAPSSKSTSGGTAALGCLVKDYFPEPVTVSWNSGALTSGVHTFPAVLQSSGLYSLSSVVTVPSSSLGTQTYICNVNHKPSNTKVDKKVEPKSCDKTHTCPPCPAPELLGGPSVFLFPPKPKDTLMISRTPEVTCVVVDVSHEDPEVKFNWYVDGVEVHNAKTKPREEQYNSTYRVVSVLTVLHQDWLNGKEYKCKVSNKALPAPIEKTISKAKGQPREPQVYTLPPSRDELTKNQVSLTCLVKGFYPSDIAVEWESNGQPENNYKTTPPVLDSDGSFFLYSKLTVDKSRWQQGNVFSCSVMHEALHNHYTQKSLSLSPGKQSVLTQPPSASGTPGQRVTISCSGSSSNIGNNDVNWYQQLPGTAPKLLIYADNQRPSGVPDRFSGSKSGTSASLAISGLRSEDEADYYCATWDASLSAYVFGGGTKLTVLRTVAAPSVFIFPPSDEQLKSGTASVVCLLNNFYPREAKVQWKVDNALQSGNSQESVTEQDSKDSTYSLSSTLTLSKADYEKHKVYACEVTHQGLSSPVTKSFNRGECF

SEQ ID NO: 33 - protein, 25 aa, synthetic construct
EVQLLESGGGLVQPGGSLRLSCAAS

SEQ ID NO: 34 - protein, 17 aa, synthetic construct
MSWVRQAPGKGLEWVSW

SEQ ID NO: 35 - protein, 38 aa, synthetic construct
YYADSVKGRFTISRDNSKNTLYLQMNSLRAEDTAVYYC

SEQ ID NO: 36 - protein, 9 aa, synthetic construct
QGTLVTVSS

SEQ ID NO: 37 - protein, 25 aa, synthetic construct
QSVLTQPPSASGTPGQRVTISCSGS

SEQ ID NO: 38 - protein, 17 aa, synthetic construct
VSWYQQLPGTAPKLLIY

SEQ ID NO: 39 - protein, 36 aa, synthetic construct
NRPSGVPDRFSGSKSGTSASLAISGLRSEDEADYYC

SEQ ID NO: 40 - protein, 10 aa, synthetic construct
FGGGTKLTVL

SEQ ID NO: 41 - protein, 25 aa, synthetic construct
EVQLLESGGGLVQPGGSLRLSCAAS

SEQ ID NO: 42 - protein, 17 aa, synthetic construct
MSWVRQAPGKGLEWVSS

SEQ ID NO: 43 - protein, 38 aa, synthetic construct; identical to SEQ ID NO: 35

SEQ ID NO: 44 - protein, 11 aa, synthetic construct
WGQGTLVTVSS

SEQ ID NO: 45 - protein, 25 aa, synthetic construct
QSVLTQPPSASGTPGQRVTISCTGS

SEQ ID NO: 46 - protein, 17 aa, synthetic construct
VSWYQQLPGTAPKLLIY

SEQ ID NO: 47 - protein, 36 aa, synthetic construct
HRPSGVPDRFSGSKSGTSASLAISGLRSEDEADYYC

SEQ ID NO: 48 - protein, 10 aa, synthetic construct
FGGGTKLTVL

SEQ ID NO: 49 - protein, 25 aa, synthetic construct
EVQLLESGEGLVQPGGSLRLSCAAS

SEQ ID NO: 50 - protein, 17 aa, synthetic construct
MSWVRQAPGKGLEWVSG

SEQ ID NO: 51 - protein, 38 aa, synthetic construct; identical to SEQ ID NO: 35

SEQ ID NO: 52 - protein, 11 aa, synthetic construct
WGQGTLVTVSS

SEQ ID NO: 53 - protein, 25 aa, synthetic construct
QSVLTQPPSASGTPGQRVTISCTGS

SEQ ID NO: 54 - protein, 17 aa, synthetic construct
VTWYQQLPGTAPKLLIY

SEQ ID NO: 55 - protein, 36 aa, synthetic construct; identical to SEQ ID NO: 39

SEQ ID NO: 56 - protein, 10 aa, synthetic construct
FCGGTKLTVL

SEQ ID NO: 57 - protein, 25 aa, synthetic construct
EVQLLESGGGLVQPGGSLRLSCAAS

SEQ ID NO: 58 - protein, 17 aa, synthetic construct
MSWVRQAPGKGLEWVSS

SEQ ID NO: 59 - protein, 38 aa, synthetic construct; identical to SEQ ID NO: 35

SEQ ID NO: 60 - protein, 11 aa, synthetic construct
WGQGTLVTVSS

SEQ ID NO: 61 - protein, 25 aa, synthetic construct
QSVLTQPPSASGTPGQRVTISCSGS

SEQ ID NO: 62 - protein, 17 aa, synthetic construct
VNWYQQLPGTAPKLLIY

SEQ ID NO: 63 - protein, 36 aa, synthetic construct
QRPSGVPDRFSGSKSGTSASLAISGLRSEDEADYYC

SEQ ID NO: 64 - protein, 10 aa, synthetic construct
FGGGTKLTVL

SEQ ID NO: 65 - DNA, 144 bp, synthetic construct
  source 1..144: mol_type = other DNA
atggaagattttaacatggagagtgacagctttgaagatttctggaaaggtgaagatcttagtaattacagttacagctctaccctgcccccttttctactagatgccgccccatgtgaaccagaatccctggaaatcaacaag

SEQ ID NO: 66 - DNA, 144 bp, synthetic construct; identical to SEQ ID NO: 65
  source 1..144: mol_type = other DNA

SEQ ID NO: 67 - DNA, 447 bp, synthetic construct
  source 1..447: mol_type = other DNA
actctaaccatggaatggagctgggtctttctcttcttcctgtcagtaactacaggtgtcctctccgaggtgcagctgttggagtccgggggaggcttggtacagcctggggggtccctgagactctcctgtgcagcctctggattcacctttagcaattattctatgagctgggtccgccaggctccagggaaggggctggagtgggtctcatggatctattataatggtggtagtacatattacgctgattctgtaaaaggtcggttcaccatctccagagacaattccaagaacacgctgtatctgcaaatgaacagcctgagagccgaggacacggccgtgtattactgtgcgagaggtcctcgtatttgtgagattcggaagtgttattctgctaatgctatggacgtctggggccagggtacactggtcaccgtgagctca

SEQ ID NO: 68 - DNA, 420 bp, synthetic construct
  source 1..420: mol_type = other DNA
cggcacgagcagaccagcatgggcatcaagatggagacacattctcaggtctttgtatacatgttgctgtggttgtctggtgttgaaggacttcatctaatattggcaataatgctgtctcctggtaccagcagctcccaggaacggcccccaaactcctcatctatgctaatagtaatcggccaagcggggtccctgaccgattctctggctccaagtctgtgctgactcagccgccctcagcgtctgggacccccgggcagagggtcaccatctcttgtagtggctcagtctggcacctcagcctccctggccatcagtgggctccggtccgaggatgaggctgattattactgtggtacttgggatgctagcctgagtgcttatgtcttcggcggaggcaccaagctgacggtccta

SEQ ID NO: 69 - DNA, 414 bp, synthetic construct
  source 1..414: mol_type = other DNA
actctaaccatggaatggagctgggtctttctcttcttcctgtcagtaactacaggtgtcctctccgaggtgcagctgttggagtctgggggaggcttggtacagcctggggggtccctgagactctcctgtgcagcctctggattcacctttagtaattatgctatgagctgggtccgccaggctccagggaaggggctggagtgggtctcatcgatctctcctagtggtagtagtaaatattacgctgattctgtaaaaggtcggttcaccatctccagagacaattccaagaacacgctgtatctgcaaatgaacagcctgagagccgaggacacggccgtgtattactgtgcgaaacataatcggcatttcgactactggggccagggtacactggtcaccgtgagctca

SEQ ID NO: 70 - DNA, 420 bp, synthetic construct
  source 1..420: mol_type = other DNA
cggcacgagcagaccagcatgggcatcaagatggagacacattctcaggtctttgtatacatgttgctgtggttgtctggtgttgaaggacagtctgtgctgactcagccaccctcagcgtctgggacccccgggcagagggtcaccatctcttgtactggctcttcatctaatattggcagtcattatgtctcctggtaccagcagctcccaggaacggcccccaaactcctcatctatgataataatcatcggccaagcggggtccctgaccgattctctggctccaagtctggcacctcagcctccctggccatcagtgggctccggtccgaggatgaggctgattattactgtggttcttgggatgatagcctgaatgcttatgtcttcggcggaggcaccaagctgacggtccta

SEQ ID NO: 71 - DNA, 414 bp, synthetic construct
  source 1..414: mol_type = other DNA
actctaaccatggaatggagctgggtctttctcttcttcctgtcagtaactacaggtgtcctctccgaggtgcagctgttggagtctggggaaggcttggtacagcctggggggtccctgagactctcctgtgcagcctctggattcacctttagcaattattctatgagctgggtccgccaggctccagggaaggggctggagtgggtctcagggatctcttctggtggtggtagtaaatattacgctgattctgtaaaaggtcggttcaccatctccagagacaattccaagaacacgctgtatctgcaaatgaacagcctgagagccgaggacacggccgtgtattactgtgcgagacaggcgactgctttcgactactggggccagggtacactggtcaccgtgagctca

SEQ ID NO: 72 - DNA, 420 bp, synthetic construct
  source 1..420: mol_type = other DNA
cggcacgagcagaccagcatgggcatcaagatggagacacattctcaggtctttgtatacatgttgctgtggttgtctggtgttgaaggacagtctgtgctgactcagccaccctcagcgtctgggacccccgggcagagggtcaccatctcttgtactggctcttcatctaatattggcaataattctgtcacctggtaccagcagctcccaggaacggcccccaaactcctcatctattctgatagtaatcggccaagcggggtccctgaccgattctctggctccaagtctggcacctcagcctccctggccatcagtgggctccggtccgaggatgaggctgattattactgtggtacttgggatgatagcctgagtgcttatgtcttcggcggaggcaccaagctgacggtccta

SEQ ID NO: 73 - DNA, 447 bp, synthetic construct
  source 1..447: mol_type = other DNA
actctaaccatggaatggagctgggtctttctcttcttcctgtcagtaactacaggtgtcctctccgaggtgcagctgttggagtctgggggaggcttggtacagcctggggggtccctgagactctcctgtgcagcctctggattcacctttagcggttatcctatgagctgggtccgccaggctccagggaaggggctggagtgggtctcatcgatctcttctagtggtggtaatacatattacgctgattctgtaaaaggtcggttcaccatctccagagacaattccaagaacacgctgtatctgcaaatgaacagcctgagagccgaggacacggccgtgtattactgtgcgagatttggtattcatcatccggatagggcgttgtattatgctaatgctatggacgtctggggccagggtacactggtcaccgtgagctca

SEQ ID NO: 74 - DNA, 420 bp, synthetic construct
  source 1..420: mol_type = other DNA
cggcacgagcagaccagcatgggcatcaagatggagacacattctcaggtctttgtatacatgttgctgtggttgtctggtgttgaaggacagtctgtgctgactcagccaccctcagcgtctgggacccccgggcagagggtcaccatctcttgtagtggctcttcatctaatattggcaataatgatgtcaactggtaccagcagctcccaggaacggcccccaaactcctcatctatgctgataatcagcggccaagcggggtccctgaccgattctctggctccaagtctggcacctcagcctccctggccatcagtgggctccggtccgaggatgaggctgattattactgtgctacttgggatgctagcctgagtgcttatgtcttcggcggaggcaccaagctgacggtccta